European Patent Application EP 4 600 272 A1, published August 13, 2025. Title: TREATMENT OF CHRONIC HEPATITIS B BASED ON INTERFERON SYNERGISTIC IMMUNE CHECKPOINT BLOCKING ANTIBODY. Applicant: IMMUNELOGIC THERAPEUTICS, INC. Application EP 23871010.7, filed September 28, 2023. The sequence listing filed with the application follows.

SEQUENCE LISTING (26 sequences)

SEQ ID NO: 1 - protein, 411 aa, synthetic construct
CDLPHTYNLGNKRALTVLEEMRRLPPLSCLKDRKDFGFPLEKVDNQQIQKAQAILVLRDLTQQILNLFTSKDLSATWNATLLDSFCNDLHQQLNDLKACVMQEPPLTQEDSLLAVRTYFHRITVYLRKKKHSLCAWEVIRAEVWRALSSSTNLLARLSEEKESGGGGSGGGGSGGGGSGGGGRTDKTHTCPPCPAPELLGGPSVFLFPPKPKDTLMISRTPEVTCVVVDVSHEDPEVKFNWYVDGVEVHNAKTKPREEQYNSTYRVVSVLTVLHQDWLNGKEYKCKVSNKALPAPIEKTISKAKGQPREPQVYTLPPCRDELTKNQVSLWCLVKGFYPSDIAVEWESNGQPENNYKTTPPVLDSDGSFFLYSALTVDKSRWQQGNVFSCSVMHEALHNHYTQKSLSLSPGK

SEQ ID NO: 2 - DNA, 1233 bp, synthetic construct
  source 1..1233: mol_type = other DNA
tgtgacctgcctcacacttataacctcgggaacaagagggccttgacagtcctggaagaaatgagaagactcccccctctttcctgcctgaaggacaggaaggattttggattccccttggagaaggtggataaccaacagatccagaaggctcaagccatccttgtgctaagagatcttacccagcagattttgaacctcttcacatcaaaagacttgtctgctacttggaatgcaactctactagactcattctgcaatgacctccatcagcagctcaatgacctcaaagcctgtgtgatgcaggaacctcctctgacccaggaagactccctgctggctgtgaggacatacttccacaggatcactgtgtacctgagaaagaagaaacacagcctctgtgcctgggaggtgatcagagcagaagtctggagagccctctcttcctcaaccaacttgctggcaagactgagtgaggagaaggagagtggcggtggtggctccggcggtggtggctccggcggtggtggctccggcggtggtggccgtacggacaaaactcacacatgcccaccgtgcccagctccggaactcctgggcggaccgtcagtcttcctcttccccccaaaacccaaggacaccctcatgatctcccggacccctgaggtcacatgcgtggtggtggacgtgagccacgaagaccctgaggtcaagttcaactggtacgtggacggcgtggaggtgcataatgccaagacaaagccgcgggaggagcagtacaacagcacgtaccgtgtggtcagcgtcctcaccgtcctgcaccaggactggctgaatggcaaggagtacaagtgcaaggtctccaacaaagccctcccagcccccatcgagaaaaccatctccaaagccaaagggcagccccgagaaccacaggtgtacaccctgcccccatgtcgggatgagctgaccaagaaccaggtcagcctgtggtgcctggtcaaaggcttctatcccagcgacatcgccgtggagtgggagagcaatgggcagccggagaacaactacaagaccacgcctcccgtgttggactccgacggctccttcttcctctacagcgcgctcaccgtggacaagagcaggtggcagcaggggaacgtcttctcatgctccgtgatgcatgaggctctgcacaaccactacacgcagaagagcctctccctgtctccgggtaaa

SEQ ID NO: 3 - protein, 215 aa, synthetic construct
DIQMTQSPSSLSASVGDRVTITCRASQDVSTAVAWYQQKPGKAPKLLIYSASFLYSGVPSRFSGSGSGTDFTLTISSLQPEDFATYYCQQYLYHPATFGQGTKVEIKRRTVAAPSVFIFPPSDEQLKSGTASVVCLLNNFYPREAKVQWKVDNALQSGNSQESVTEQDSKDSTYSLSSTLTLSKADYEKHKVYACEVTHQGLSSPVTKSFNRGEC

SEQ ID NO: 4 - DNA, 645 bp, synthetic construct
  source 1..645: mol_type = other DNA
gacatccagatgacccagagccccagcagcctgagcgccagcgtgggcgacagagtgaccatcacctgcagagccagccaggacgtgagcaccgccgtggcctggtaccagcagaagcccggcaaggcccccaagctgctgatctacagcgccagcttcctgtacagcggcgtgcccagcagattcagcggcagcggcagcggcaccgacttcaccctgaccatcagcagcctgcagcccgaggacttcgccacctactactgccagcagtacctgtaccaccccgccaccttcggccagggcaccaaggtggagatcaagagacgtacggtggctgcaccatctgtcttcatcttcccgccatctgatgagcagttgaaatctggtaccgctagcgttgtgtgcctgctgaataacttttatccacgggaggctaaggtgcagtggaaagtggacaatgccctccagagcggaaatagccaagagtccgttaccgaacaggactctaaagactctacatactccctgtcctccacactgaccctctccaaggccgactatgagaaacacaaggtttacgcatgcgaggtcacacaccagggactctcctctcccgtgaccaagagcttcaaccggggagaatgc

SEQ ID NO: 5 - protein, 448 aa, synthetic construct
EVQLVESGGGLVQPGGSLRLSCAASGFTFSDSWIHWVRQAPGKGLEWVAWISPYGGSTYYADSVKGRFTISADTSKNTAYLQMNSLRAEDTAVYYCARRHWPGGFDYWGQGTLVTVSAASTKGPSVFPLAPSSKSTSGGTAALGCLVKDYFPEPVTVSWNSGALTSGVHTFPAVLQSSGLYSLSSVVTVPSSSLGTQTYICNVNHKPSNTKVDKRVEPKSCDKTHTCPPCPAPELLGGPSVFLFPPKPKDTLMISRTPEVTCVVVDVSHEDPEVKFNWYVDGVEVHNAKTKPREEQYNSTYRVVSVLTVLHQDWLNGKEYKCKVSNKALPAPIEKTISKAKGQPREPQVCTLPPSRDELTKNQVSLSCAVKGFYPSDIAVEWESNGQPENNYKTTPPVLDSDGSFKLVSKLTVDKSRWQQGNVFSCSVMHEALHNHYTQKSLSLSPGK

SEQ ID NO: 6 - DNA, 1344 bp, synthetic construct
  source 1..1344: mol_type = other DNA
gaggtgcagctggtggagagcggcggcggcctggtgcagcccggcggcagcctgagactgagctgcgccgccagcggcttcaccttcagcgacagctggatccactgggtgagacaggcccccggcaagggcctggagtgggtggcctggatcagcccctacggcggcagcacctactacgccgacagcgtgaagggcagattcaccatcagcgccgacaccagcaagaacaccgcctacctgcagatgaacagcctgagagccgaggacaccgccgtgtactactgcgccagaagacactggcccggcggcttcgactactggggccagggcaccctggtgaccgtgagcgccgccagcactaaggggccctctgtgtttccactcgccccttctagcaaaagcacttccggaggaactgccgctctgggctgtctggtgaaagattacttccccgaaccagtcactgtgtcatggaactctggagcactgacatctggagttcacacctttcctgctgtgctgcagagttctggactgtactccctgtcatctgtggtcaccgtgccatcttcatctctggggacccagacctacatctgtaacgtgaaccacaaaccctccaacacaaaagtcgacaaacgagtcgaaccaaaatcttgtgacaaaacccacacatgcccaccttgtcccgcccctgaactcctgggcggaccgtcagtcttcctcttccccccaaaacccaaggacaccctcatgatctcccggacccctgaggtcacatgcgtggtggtggacgtgagccacgaagaccctgaggtcaagttcaactggtacgtggacggcgtggaggtgcataatgccaagacaaagccgcgggaggagcagtacaacagcacgtaccgtgtggtcagcgtcctcaccgtcctgcaccaggactggctgaatggcaaggagtacaagtgcaaggtctccaacaaagccctcccagcccccatcgagaaaaccatctccaaagccaaagggcagccccgagaaccacaggtgtgtaccctgcccccatcccgggatgagctgaccaagaaccaggtcagcctgagttgcgcggtcaaaggcttctatcccagcgacatcgccgtggagtgggagagcaatgggcagccggagaacaactacaagaccacgcctcccgtgttggactccgacggctccttcaagctcgtcagcaagctcaccgtggacaagagcaggtggcagcaggggaacgtcttctcatgctccgtgatgcatgaggctctgcacaaccactacacgcagaagagcctctccctgtctccgggtaaa

SEQ ID NO: 7 - protein, 638 aa, synthetic construct
CDLPHTYNLGNKRALTVLEEMRRLPPLSCLKDRKDFGFPLEKVDNQQIQKAQAILVLRDLTQQILNLFTSKDLSATWNATLLDSFCNDLHQQLNDLKACVMQEPPLTQEDSLLAVRTYFHRITVYLRKKKHSLCAWEVIRAEVWRALSSSTNLLARLSEEKESGGGGSGGGGSGGGGSGGGGRTEVQLVESGGGLVQPGGSLRLSCAASGFTFSDSWIHWVRQAPGKGLEWVAWISPYGGSTYYADSVKGRFTISADTSKNTAYLQMNSLRAEDTAVYYCARRHWPGGFDYWGQGTLVTVSAASTKGPSVFPLAPSSKSTSGGTAALGCLVKDYFPEPVTVSWNSGALTSGVHTFPAVLQSSGLYSLSSVVTVPSSSLGTQTYICNVNHKPSNTKVDKRVEPKSCFEEPKSCDKTHTCPPCPAPELLGGPSVFLFPPKPKDQLMISRTPEVTCVVVDVSHEDPEVKFNWYVDGVEVHNAKTKPREEQYNSTYRVVSVLTVLHQDWLNGKEYKCKVSNKALPAPIEKTISKAKGQPREPQVYTLPPSRDELTKNQVSLTCLVKGFYPSDIAVEWESNGQPENNYKTTPPVLDSDGSFLYSKLTVDKSRWQQGNVFSCSVLHEALHNHYTQKSLSLSPGK

SEQ ID NO: 8 - DNA, 1914 bp, synthetic construct
  source 1..1914: mol_type = other DNA
tgtgacctgcctcacacttataacctcgggaacaagagggccttgacagtcctggaagaaatgagaagactcccccctctttcctgcctgaaggacaggaaggattttggattccccttggagaaggtggataaccaacagatccagaaggctcaagccatccttgtgctaagagatcttacccagcagattttgaacctcttcacatcaaaagacttgtctgctacttggaatgcaactctactagactcattctgcaatgacctccatcagcagctcaatgacctcaaagcctgtgtgatgcaggaacctcctctgacccaggaagactccctgctggctgtgaggacatacttccacaggatcactgtgtacctgagaaagaagaaacacagcctctgtgcctgggaggtgatcagagcagaagtctggagagccctctcttcctcaaccaacttgctggcaagactgagtgaggagaaggagagtggcggtggtggctccggcggtggtggctccggcggtggtggctccggcggtggtggccgtacggaggtgcagctggtggagagcggcggcggcctggtgcagcccggcggcagcctgagactgagctgcgccgccagcggcttcaccttcagcgacagctggatccactgggtgagacaggcccccggcaagggcctggagtgggtggcctggatcagcccctacggcggcagcacctactacgccgacagcgtgaagggcagattcaccatcagcgccgacaccagcaagaacaccgcctacctgcagatgaacagcctgagagccgaggacaccgccgtgtactactgcgccagaagacactggcccggcggcttcgactactggggccagggcaccctggtgaccgtgagcgccgccagcactaaggggccctctgtgtttccactcgccccttctagcaaaagcacttccggaggaactgccgctctgggctgtctggtgaaagattacttccccgaaccagtcactgtgtcatggaactctggagcactgacatctggagttcacacctttcctgctgtgctgcagagttctggactgtactccctgtcatctgtggtcaccgtgccatcttcatctctggggacccagacctacatctgtaacgtgaaccacaaaccctccaacacaaaagtcgacaaacgagtcgaaccaaaatcttgtttcgaagagcccaagagctgcgacaagacccacacctgtcccccttgtcctgcccctgagctgctgggcggacccagcgtgttcctgttccccccaaagcccaaggaccagctgatgatcagccggacccccgaagtgacctgcgtggtggtggacgtgtcccacgaggaccctgaagtgaagttcaattggtacgtggacggcgtggaggtgcacaacgccaagaccaagccccgggaggaacagtacaacagcacctaccgggtggtgtccgtgctgaccgtgctgcaccaggactggctgaacggcaaagagtacaagtgcaaggtctccaacaaggccctgcctgcccccatcgaaaagaccatcagcaaggccaagggccagcccagagaaccccaggtgtacaccctgccccccagcagagatgagctgaccaagaaccaggtgtccctgacctgcctggtcaagggcttctaccccagcgatatcgccgtggagtgggagagcaacggccagcctgagaacaactacaagaccaccccccctgtgctggacagcgatggcagcttcctctacagcaaactgaccgtggacaagagccggtggcagcagggcaacgtgttcagctgcagcgtgttgcacgaggccctgcacaaccactacacccagaagtccctgagcctgagccccggcaaa

SEQ ID NO: 9 - protein, 472 aa, synthetic construct
ELDIQMTQSPSSLSASVGDRVTITCRASQDVSTAVAWYQQKPGKAPKLLIYSASFLYSGVPSRFSGSGSGTDFTLTISSLQPEDFATYYCQQYLYHPATFGQGTKVEIKRGGGGSGGGGSGGGGSEVQLVESGGGLVQPGGSLRLSCAASGFTFSDSWIHWVRQAPGKGLEWVAWISPYGGSTYYADSVKGRFTISADTSKNTAYLQMNSLRAEDTAVYYCARRHWPGGFDYWGQGTLVTVSARSDKTHTCPPCPAPELLGGPSVFLFPPKPKDTLMISRTPEVTCVVVDVSHEDPEVKFNWYVDGVEVHNAKTKPREEQYNSTYRVVSVLTVLHQDWLNGKEYKCKVSNKALPAPIEKTISKAKGQPREPQVYTLPPCRDELTKNQVSLWCLVKGFYPSDIAVEWESNGQPENNYKTTPPVLDSDGSFFLYSKLTVDKSRWQQGNVFSCSVMHEALHNHYTQKSLSLSPGK

SEQ ID NO: 10 - DNA, 1419 bp, synthetic construct
  source 1..1419: mol_type = other DNA
gagctcgacatccagatgacccagagccccagcagcctgagcgccagcgtgggcgacagagtgaccatcacctgcagagccagccaggacgtgagcaccgccgtggcctggtaccagcagaagcccggcaaggcccccaagctgctgatctacagcgccagcttcctgtacagcggcgtgcccagcagattcagcggcagcggcagcggcaccgacttcaccctgaccatcagcagcctgcagcccgaggacttcgccacctactactgccagcagtacctgtaccaccccgccaccttcggccagggcaccaaggtggagatcaagagaggcggcggcggcagcggcggcggcggcagcggcggcggcggcagcgaggtgcagctggtggagagcggcggcggcctggtgcagcccggcggcagcctgagactgagctgcgccgccagcggcttcaccttcagcgacagctggatccactgggtgagacaggcccccggcaagggcctggagtgggtggcctggatcagcccctacggcggcagcacctactacgccgacagcgtgaagggcagattcaccatcagcgccgacaccagcaagaacaccgcctacctgcagatgaacagcctgagagccgaggacaccgccgtgtactactgcgccagaagacactggcccggcggcttcgactactggggccagggcaccctggtgaccgtgagcgccagatctgacaagacccacacctgccccccctgccccgcccccgagctgctgggcggccccagcgtgttcctgttcccccccaagcccaaggacaccctgatgatcagccgcacccccgaggtgacctgcgtggtggtggacgtgagccacgaggaccccgaggtgaagttcaactggtacgtggacggcgtggaggtgcacaacgccaagaccaagccccgcgaggagcagtacaacagcacctaccgcgtggtgagcgtgctgaccgtgctgcaccaggactggctgaacggcaaggagtacaagtgcaaggtgagcaacaaggccctgcccgcccccatcgagaagaccatcagcaaggccaagggccagccccgcgagccccaggtgtacaccctgcccccctgccgcgacgagctgaccaagaaccaggtgagcctgtggtgcctggtgaagggcttctaccccagcgacatcgccgtggagtgggagagcaacggccagcccgagaacaactacaagaccaccccccccgtgctggacagcgacggcagcttcttcctgtacagcaagctgaccgtggacaagagccgctggcagcagggcaacgtgttcagctgcagcgtgatgcacgaggccctgcacaaccactacacccagaagagcctgagcctgagccccggcaagtaa

SEQ ID NO: 11 - protein, 658 aa, synthetic construct
CDLPHTYNLGNKRALTVLEEMRRLPPLSCLKDRKDFGFPLEKVDNQQIQKAQAILVLRDLTQQILNLFTSKDLSATWNATLLDSFCNDLHQQLNDLKACVMQEPPLTQEDSLLAVRTYFHRITVYLRKKKHSLCAWEVIRAEVWRALSSSTNLLARLSEEKESGGGGSGGGGSGGGGSGGGGRTDIQMTQSPSSLSASVGDRVTITCRASQDVSTAVAWYQQKPGKAPKLLIYSASFLYSGVPSRFSGSGSGTDFTLTISSLQPEDFATYYCQQYLYHPATFGQGTKVEIKRGGGGSGGGGSGGGGSEVQLVESGGGLVQPGGSLRLSCAASGFTFSDSWIHWVRQAPGKGLEWVAWISPYGGSTYYADSVKGRFTISADTSKNTAYLQMNSLRAEDTAVYYCARRHWPGGFDYWGQGTLVTVSAFEEPKSCDKTHTCPPCPAPELLGGPSVFLFPPKPKDQLMISRTPEVTCVVVDVSHEDPEVKFNWYVDGVEVHNAKTKPREEQYNSTYRVVSVLTVLHQDWLNGKEYKCKVSNKALPAPIEKTISKAKGQPREPQVYTLPPSRDELTKNQVSLTCLVKGFYPSDIAVEWESNGQPENNYKTTPPVLDSDGSFLYSKLTVDKSRWQQGNVFSCSVLHEALHNHYTQKSLSLSPGK

SEQ ID NO: 12 - DNA, 1974 bp, synthetic construct
  source 1..1974: mol_type = other DNA
tgtgacctgcctcacacttataacctcgggaacaagagggccttgacagtcctggaagaaatgagaagactcccccctctttcctgcctgaaggacaggaaggattttggattccccttggagaaggtggataaccaacagatccagaaggctcaagccatccttgtgctaagagatcttacccagcagattttgaacctcttcacatcaaaagacttgtctgctacttggaatgcaactctactagactcattctgcaatgacctccatcagcagctcaatgacctcaaagcctgtgtgatgcaggaacctcctctgacccaggaagactccctgctggctgtgaggacatacttccacaggatcactgtgtacctgagaaagaagaaacacagcctctgtgcctgggaggtgatcagagcagaagtctggagagccctctcttcctcaaccaacttgctggcaagactgagtgaggagaaggagagtggcggtggtggctccggcggtggtggctccggcggtggtggctccggcggtggtggccgtacggacatccagatgacccagagccccagcagcctgagcgccagcgtgggcgacagagtgaccatcacctgcagagccagccaggacgtgagcaccgccgtggcctggtaccagcagaagcccggcaaggcccccaagctgctgatctacagcgccagcttcctgtacagcggcgtgcccagcagattcagcggcagcggcagcggcaccgacttcaccctgaccatcagcagcctgcagcccgaggacttcgccacctactactgccagcagtacctgtaccaccccgccaccttcggccagggcaccaaggtggagatcaagagaggcggcggcggcagcggcggcggcggcagcggcggcggcggcagcgaggtgcagctggtggagagcggcggcggcctggtgcagcccggcggcagcctgagactgagctgcgccgccagcggcttcaccttcagcgacagctggatccactgggtgagacaggcccccggcaagggcctggagtgggtggcctggatcagcccctacggcggcagcacctactacgccgacagcgtgaagggcagattcaccatcagcgccgacaccagcaagaacaccgcctacctgcagatgaacagcctgagagccgaggacaccgccgtgtactactgcgccagaagacactggcccggcggcttcgactactggggccagggcaccctggtgaccgtgagcgccttcgaagagcccaagagctgcgacaagacccacacctgtcccccttgtcctgcccctgagctgctgggcggacccagcgtgttcctgttccccccaaagcccaaggaccagctgatgatcagccggacccccgaagtgacctgcgtggtggtggacgtgtcccacgaggaccctgaagtgaagttcaattggtacgtggacggcgtggaggtgcacaacgccaagaccaagccccgggaggaacagtacaacagcacctaccgggtggtgtccgtgctgaccgtgctgcaccaggactggctgaacggcaaagagtacaagtgcaaggtctccaacaaggccctgcctgcccccatcgaaaagaccatcagcaaggccaagggccagcccagagaaccccaggtgtacaccctgccccccagcagagatgagctgaccaagaaccaggtgtccctgacctgcctggtcaagggcttctaccccagcgatatcgccgtggagtgggagagcaacggccagcctgagaacaactacaagaccaccccccctgtgctggacagcgatggcagcttcctctacagcaaactgaccgtggacaagagccggtggcagcagggcaacgtgttcagctgcagcgtgttgcacgaggccctgcacaaccactacacccagaagtccctgagcctgagccccggcaaa

SEQ ID NO: 13 - protein, 415 aa, synthetic construct
CDLPHTYNLGNKRALTVLEEMRRLPPLSCLKDRKDFGFPLEKVDNQQIQKAQAILVLRDLTQQILNLFTSKDLSATWNATLLDSFCNDLHQQLNDLKACVMQEPPLTQEDSLLAVRTYFHRITVYLRKKKHSLCAWEVIRAEVWRALSSSTNLLARLSEEKESGGGGSGGGGSGGGGSGGGGRTEPKSCDKTHTCPPCPAPELLGGPSVFLFPPKPKDQLMISRTPEVTCVVVDVSHEDPEVKFNWYVDGVEVHNAKTKPREEQYNSTYRVVSVLTVLHQDWLNGKEYKCKVSNKALPAPIEKTISKAKGQPREPQVYTLPPSRDELTKNQVSLTCLVKGFYPSDIAVEWESNGQPENNYKTTPPVLDSDGSFLYSKLTVDKSRWQQGNVFSCSVLHEALHNHYTQKSLSLSPGK

SEQ ID NO: 14 - DNA, 1245 bp, synthetic construct
  source 1..1245: mol_type = other DNA
tgtgacctgcctcacacttataacctcgggaacaagagggccttgacagtcctggaagaaatgagaagactcccccctctttcctgcctgaaggacaggaaggattttggattccccttggagaaggtggataaccaacagatccagaaggctcaagccatccttgtgctaagagatcttacccagcagattttgaacctcttcacatcaaaagacttgtctgctacttggaatgcaactctactagactcattctgcaatgacctccatcagcagctcaatgacctcaaagcctgtgtgatgcaggaacctcctctgacccaggaagactccctgctggctgtgaggacatacttccacaggatcactgtgtacctgagaaagaagaaacacagcctctgtgcctgggaggtgatcagagcagaagtctggagagccctctcttcctcaaccaacttgctggcaagactgagtgaggagaaggagagtggcggtggtggctccggcggtggtggctccggcggtggtggctccggcggtggtggccgtacggagcccaagagctgcgacaagacccacacctgtcccccttgtcctgcccctgagctgctgggcggacccagcgtgttcctgttccccccaaagcccaaggaccagctgatgatcagccggacccccgaagtgacctgcgtggtggtggacgtgtcccacgaggaccctgaagtgaagttcaattggtacgtggacggcgtggaggtgcacaacgccaagaccaagccccgggaggaacagtacaacagcacctaccgggtggtgtccgtgctgaccgtgctgcaccaggactggctgaacggcaaagagtacaagtgcaaggtctccaacaaggccctgcctgcccccatcgaaaagaccatcagcaaggccaagggccagcccagagaaccccaggtgtacaccctgccccccagcagagatgagctgaccaagaaccaggtgtccctgacctgcctggtcaagggcttctaccccagcgatatcgccgtggagtgggagagcaacggccagcctgagaacaactacaagaccaccccccctgtgctggacagcgatggcagcttcctctacagcaaactgaccgtggacaagagccggtggcagcagggcaacgtgttcagctgcagcgtgttgcacgaggccctgcacaaccactacacccagaagtccctgagcctgagccccggcaaa

SEQ ID NO: 15 - protein, 454 aa, synthetic construct
EVQLVESGGGLVQPGGSLRLSCAASGFTFSDSWIHWVRQAPGKGLEWVAWISPYGGSTYYADSVKGRFTISADTSKNTAYLQMNSLRAEDTAVYYCARRHWPGGFDYWGQGTLVTVSAASTKGPSVFPLAPSSKSTSGGTAALGCLVKDYFPEPVTVSWNSGALTSGVHTFPAVLQSSGLYSLSSVVTVPSSSLGTQTYICNVNHKPSNTKVDKRVEPKSCRTEPKSCDKTHTCPPCPAPELLGGPSVFLFPPKPKDQLMISRTPEVTCVVVDVSHEDPEVKFNWYVDGVEVHNAKTKPREEQYNSTYRVVSVLTVLHQDWLNGKEYKCKVSNKALPAPIEKTISKAKGQPREPQVYTLPPSRDELTKNQVSLTCLVKGFYPSDIAVEWESNGQPENNYKTTPPVLDSDGSFLYSKLTVDKSRWQQGNVFSCSVLHEALHNHYTQKSLSLSPGK

SEQ ID NO: 16 - DNA, 1362 bp, synthetic construct
  source 1..1362: mol_type = other DNA
gaggtgcagctggtggagagcggcggcggcctggtgcagcccggcggcagcctgagactgagctgcgccgccagcggcttcaccttcagcgacagctggatccactgggtgagacaggcccccggcaagggcctggagtgggtggcctggatcagcccctacggcggcagcacctactacgccgacagcgtgaagggcagattcaccatcagcgccgacaccagcaagaacaccgcctacctgcagatgaacagcctgagagccgaggacaccgccgtgtactactgcgccagaagacactggcccggcggcttcgactactggggccagggcaccctggtgaccgtgagcgccgccagcactaaggggccctctgtgtttccactcgccccttctagcaaaagcacttccggaggaactgccgctctgggctgtctggtgaaagattacttccccgaaccagtcactgtgtcatggaactctggagcactgacatctggagttcacacctttcctgctgtgctgcagagttctggactgtactccctgtcatctgtggtcaccgtgccatcttcatctctggggacccagacctacatctgtaacgtgaaccacaaaccctccaacacaaaagtcgacaaacgagtcgaaccaaaatcttgtcgtacggagcccaagagctgcgacaagacccacacctgtcccccttgtcctgcccctgagctgctgggcggacccagcgtgttcctgttccccccaaagcccaaggaccagctgatgatcagccggacccccgaagtgacctgcgtggtggtggacgtgtcccacgaggaccctgaagtgaagttcaattggtacgtggacggcgtggaggtgcacaacgccaagaccaagccccgggaggaacagtacaacagcacctaccgggtggtgtccgtgctgaccgtgctgcaccaggactggctgaacggcaaagagtacaagtgcaaggtctccaacaaggccctgcctgcccccatcgaaaagaccatcagcaaggccaagggccagcccagagaaccccaggtgtacaccctgccccccagcagagatgagctgaccaagaaccaggtgtccctgacctgcctggtcaagggcttctaccccagcgatatcgccgtggagtgggagagcaacggccagcctgagaacaactacaagaccaccccccctgtgctggacagcgatggcagcttcctctacagcaaactgaccgtggacaagagccggtggcagcagggcaacgtgttcagctgcagcgtgttgcacgaggccctgcacaaccactacacccagaagtccctgagcctgagccccggcaaa

SEQ ID NO: 17 - protein, 474 aa, synthetic construct
DIQMTQSPSSLSASVGDRVTITCRASQDVSTAVAWYQQKPGKAPKLLIYSASFLYSGVPSRFSGSGSGTDFTLTISSLQPEDFATYYCQQYLYHPATFGQGTKVEIKRGGGGSGGGGSGGGGSEVQLVESGGGLVQPGGSLRLSCAASGFTFSDSWIHWVRQAPGKGLEWVAWISPYGGSTYYADSVKGRFTISADTSKNTAYLQMNSLRAEDTAVYYCARRHWPGGFDYWGQGTLVTVSARTEPKSCDKTHTCPPCPAPELLGGPSVFLFPPKPKDQLMISRTPEVTCVVVDVSHEDPEVKFNWYVDGVEVHNAKTKPREEQYNSTYRVVSVLTVLHQDWLNGKEYKCKVSNKALPAPIEKTISKAKGQPREPQVYTLPPSRDELTKNQVSLTCLVKGFYPSDIAVEWESNGQPENNYKTTPPVLDSDGSFLYSKLTVDKSRWQQGNVFSCSVLHEALHNHYTQKSLSLSPGK

SEQ ID NO: 18 - DNA, 1422 bp, synthetic construct
  source 1..1422: mol_type = other DNA
gacatccagatgacccagagccccagcagcctgagcgccagcgtgggcgacagagtgaccatcacctgcagagccagccaggacgtgagcaccgccgtggcctggtaccagcagaagcccggcaaggcccccaagctgctgatctacagcgccagcttcctgtacagcggcgtgcccagcagattcagcggcagcggcagcggcaccgacttcaccctgaccatcagcagcctgcagcccgaggacttcgccacctactactgccagcagtacctgtaccaccccgccaccttcggccagggcaccaaggtggagatcaagagaggcggcggcggcagcggcggcggcggcagcggcggcggcggcagcgaggtgcagctggtggagagcggcggcggcctggtgcagcccggcggcagcctgagactgagctgcgccgccagcggcttcaccttcagcgacagctggatccactgggtgagacaggcccccggcaagggcctggagtgggtggcctggatcagcccctacggcggcagcacctactacgccgacagcgtgaagggcagattcaccatcagcgccgacaccagcaagaacaccgcctacctgcagatgaacagcctgagagccgaggacaccgccgtgtactactgcgccagaagacactggcccggcggcttcgactactggggccagggcaccctggtgaccgtgagcgcccgtacggagcccaagagctgcgacaagacccacacctgtcccccttgtcctgcccctgagctgctgggcggacccagcgtgttcctgttccccccaaagcccaaggaccagctgatgatcagccggacccccgaagtgacctgcgtggtggtggacgtgtcccacgaggaccctgaagtgaagttcaattggtacgtggacggcgtggaggtgcacaacgccaagaccaagccccgggaggaacagtacaacagcacctaccgggtggtgtccgtgctgaccgtgctgcaccaggactggctgaacggcaaagagtacaagtgcaaggtctccaacaaggccctgcctgcccccatcgaaaagaccatcagcaaggccaagggccagcccagagaaccccaggtgtacaccctgccccccagcagagatgagctgaccaagaaccaggtgtccctgacctgcctggtcaagggcttctaccccagcgatatcgccgtggagtgggagagcaacggccagcctgagaacaactacaagaccaccccccctgtgctggacagcgatggcagcttcctctacagcaaactgaccgtggacaagagccggtggcagcagggcaacgtgttcagctgcagcgtgttgcacgaggccctgcacaaccactacacccagaagtccctgagcctgagccccggcaaa

SEQ ID NO: 19 - protein, 411 aa, synthetic construct
CDLPHTYNLGNKRALTVLEEMRRLPPLSCLKDRKDFGFPLEKVDNQQIQKAQAILVLRDLTQQILNLFTSKDLSATWNATLLDSFCNDLHQQLNDLKACVMQEPPLTQEDSLLAVRTYFHRITVYLRKKKHSLCAWEVIRAEVWRALSSSTNLLARLSEEKESGGGGSGGGGSGGGGSGGGGRTDKTHTCPPCPAPEAAGGPSVFLFPPKPKDTLMISRTPEVTCVVVDVSHEDPEVKFNWYVDGVEVHNAKTKPREEQYNSTYRVVSVLTVLHQDWLNGKEYKCKVSNKALGAPIEKTISKAKGQPREPQVYTLPPCRDELTKNQVSLWCLVKGFYPSDIAVEWESNGQPENNYKTTPPVLDSDGSFFLYSALTVDKSRWQQGNVFSCSVMHEALHNHYTQKSLSLSPGK

SEQ ID NO: 20 - DNA, 1233 bp, synthetic construct
  source 1..1233: mol_type = other DNA
tgtgacctgcctcacacttataacctcgggaacaagagggccttgacagtcctggaagaaatgagaagactcccccctctttcctgcctgaaggacaggaaggattttggattccccttggagaaggtggataaccaacagatccagaaggctcaagccatccttgtgctaagagatcttacccagcagattttgaacctcttcacatcaaaagacttgtctgctacttggaatgcaactctactagactcattctgcaatgacctccatcagcagctcaatgacctcaaagcctgtgtgatgcaggaacctcctctgacccaggaagactccctgctggctgtgaggacatacttccacaggatcactgtgtacctgagaaagaagaaacacagcctctgtgcctgggaggtgatcagagcagaagtctggagagccctctcttcctcaaccaacttgctggcaagactgagtgaggagaaggagagtggcggtggtggctccggcggtggtggctccggcggtggtggctccggcggtggtggccgtacggacaaaacccacacatgcccaccttgtcccgcccctgaagccgcaggcggaccgtcagtcttcctcttccccccaaaacccaaggacaccctcatgatctcccggacccctgaggtcacatgcgtggtggtggacgtgagccacgaagaccctgaggtcaagttcaactggtacgtggacggcgtggaggtgcataatgccaagacaaagccgcgggaggagcagtacaacagcacgtaccgtgtggtcagcgtcctcaccgtcctgcaccaggactggctgaatggcaaggagtacaagtgcaaggtctccaacaaagccctcggagcccccatcgagaaaaccatctccaaagccaaagggcagccccgagaaccacaggtgtacaccctgcccccatgtcgggatgagctgaccaagaaccaggtcagcctgtggtgcctggtcaaaggcttctatcccagcgacatcgccgtggagtgggagagcaatgggcagccggagaacaactacaagaccacgcctcccgtgttggactccgacggctccttcttcctctacagcgcgctcaccgtggacaagagcaggtggcagcaggggaacgtcttctcatgctccgtgatgcatgaggctctgcacaaccactacacgcagaagagcctctccctgtctccgggtaaa

SEQ ID NO: 21 - protein, 448 aa, synthetic construct
EVQLVESGGGLVQPGGSLRLSCAASGFTFSDSWIHWVRQAPGKGLEWVAWISPYGGSTYYADSVKGRFTISADTSKNTAYLQMNSLRAEDTAVYYCARRHWPGGFDYWGQGTLVTVSAASTKGPSVFPLAPSSKSTSGGTAALGCLVKDYFPEPVTVSWNSGALTSGVHTFPAVLQSSGLYSLSSVVTVPSSSLGTQTYICNVNHKPSNTKVDKRVEPKSCDKTHTCPPCPAPEAAGGPSVFLFPPKPKDTLMISRTPEVTCVVVDVSHEDPEVKFNWYVDGVEVHNAKTKPREEQYNSTYRVVSVLTVLHQDWLNGKEYKCKVSNKALGAPIEKTISKAKGQPREPQVCTLPPSRDELTKNQVSLSCAVKGFYPSDIAVEWESNGQPENNYKTTPPVLDSDGSFKLVSKLTVDKSRWQQGNVFSCSVMHEALHNHYTQKSLSLSPGK

SEQ ID NO: 22 - DNA, 1344 bp, synthetic construct
  source 1..1344: mol_type = other DNA
gaggtgcagctggtggagagcggcggcggcctggtgcagcccggcggcagcctgagactgagctgcgccgccagcggcttcaccttcagcgacagctggatccactgggtgagacaggcccccggcaagggcctggagtgggtggcctggatcagcccctacggcggcagcacctactacgccgacagcgtgaagggcagattcaccatcagcgccgacaccagcaagaacaccgcctacctgcagatgaacagcctgagagccgaggacaccgccgtgtactactgcgccagaagacactggcccggcggcttcgactactggggccagggcaccctggtgaccgtgagcgccgccagcactaaggggccctctgtgtttccactcgccccttctagcaaaagcacttccggaggaactgccgctctgggctgtctggtgaaagattacttccccgaaccagtcactgtgtcatggaactctggagcactgacatctggagttcacacctttcctgctgtgctgcagagttctggactgtactccctgtcatctgtggtcaccgtgccatcttcatctctggggacccagacctacatctgtaacgtgaaccacaaaccctccaacacaaaagtcgacaaacgagtcgaaccaaaatcttgtgacaaaacccacacatgcccaccttgtcccgcccctgaagccgcaggcggaccgtcagtcttcctcttccccccaaaacccaaggacaccctcatgatctcccggacccctgaggtcacatgcgtggtggtggacgtgagccacgaagaccctgaggtcaagttcaactggtacgtggacggcgtggaggtgcataatgccaagacaaagccgcgggaggagcagtacaacagcacgtaccgtgtggtcagcgtcctcaccgtcctgcaccaggactggctgaatggcaaggagtacaagtgcaaggtctccaacaaagccctcggagcccccatcgagaaaaccatctccaaagccaaagggcagccccgagaaccacaggtgtgtaccctgcccccatcccgggatgagctgaccaagaaccaggtcagcctgagttgcgcggtcaaaggcttctatcccagcgacatcgccgtggagtgggagagcaatgggcagccggagaacaactacaagaccacgcctcccgtgttggactccgacggctccttcaagctcgtcagcaagctcaccgtggacaagagcaggtggcagcaggggaacgtcttctcatgctccgtgatgcatgaggctctgcacaaccactacacgcagaagagcctctccctgtctccgggtaaa

SEQ ID NO: 23 - protein, 409 aa, synthetic construct
CDLPQTHSLGSRRTLMLLAQMRRISLFSCLKDRHDFGFPQEEFGNQFQKAETIPVLHEMIQQIFNLFSTKDSSAAWDETLLDKFYTELYQQLNDLEACVIQGVGVTETPLMKEDSILAVRKYFRRITLYLKEKKYSPCAWEVVRAEIMRSFSLSTNLQESLRSKEGGGGSGGGGSGGGGSRTDKTHTCPPCPAPELLGGPSVFLFPPKPKDTLMISRTPEVTCVVVDVSHEDPEVKFNWYVDGVEVHNAKTKPREEQYNSTYRVVSVLTVLHQDWLNGKEYKCKVSNKALPAPIEKTISKAKGQPREPQVYTLPPCRDELTKNQVSLWCLVKGFYPSDIAVEWESNGQPENNYKTTPPVLDSDGSFFLYSALTVDKSRWQQGNVFSCSVMHEALHNHYTQKSLSLSPGK

SEQ ID NO: 24 - DNA, 1227 bp, synthetic construct
  source 1..1227: mol_type = other DNA
tgcgatttaccccagacacactctttaggctctcgtaggaccctcatgctgctggcccagatgaggaggatctctttattctcttgtttaaaggacagacacgacttcggcttcccccaagaagagttcggcaaccagttccagaaggctgagaccatccccgtgctgcacgagatgatccagcagatcttcaatttatttagcaccaaggactccagcgccgcttgggatgagactttactggacaagttctacaccgaactgtaccagcagctgaacgatttagaggcttgtgtgatccaaggtgtgggagtgaccgagacccctctgatgaaggaggactccattttagccgtgaggaagtactttcgtaggatcaccctctacctcaaggagaagaagtacagcccttgcgcttgggaggtggtgagggctgagattatgaggagcttctctttatccaccaatctgcaagaatctttaaggtccaaggaaggcggaggcggatcaggcggcggtggatctgggggtggcggatctcgtacggacaaaacccacacatgcccaccttgtcccgcccctgaactcctgggcggaccgtcagtcttcctcttccccccaaaacccaaggacaccctcatgatctcccggacccctgaggtcacatgcgtggtggtggacgtgagccacgaagaccctgaggtcaagttcaactggtacgtggacggcgtggaggtgcataatgccaagacaaagccgcgggaggagcagtacaacagcacgtaccgtgtggtcagcgtcctcaccgtcctgcaccaggactggctgaatggcaaggagtacaagtgcaaggtctccaacaaagccctcccagcccccatcgagaaaaccatctccaaagccaaagggcagccccgagaaccacaggtgtacaccctgcccccatgtcgggatgagctgaccaagaaccaggtcagcctgtggtgcctggtcaaaggcttctatcccagcgacatcgccgtggagtgggagagcaatgggcagccggagaacaactacaagaccacgcctcccgtgttggactccgacggctccttcttcctctacagcgcgctcaccgtggacaagagcaggtggcagcaggggaacgtcttctcatgctccgtgatgcatgaggctctgcacaaccactacacgcagaagagcctctccctgtctccgggtaaa

SEQ ID NO: 25 - protein, 409 aa, synthetic construct
CDLPQTHSLGSRRTLMLLAQMRRISLFSCLKDRHDFGFPQEEFGNQFQKAETIPVLHEMIQQIFNLFSTKDSSAAWDETLLDKFYTELYQQLNDLEACVIQGVGVTETPLMKEDSILAVRKYFRRITLYLKEKKYSPCAWEVVRAEIMRSFSLSTNLQESLRSKEGGGGSGGGGSGGGGSRTDKTHTCPPCPAPEAAGGPSVFLFPPKPKDTLMISRTPEVTCVVVDVSHEDPEVKFNWYVDGVEVHNAKTKPREEQYNSTYRVVSVLTVLHQDWLNGKEYKCKVSNKALGAPIEKTISKAKGQPREPQVYTLPPCRDELTKNQVSLWCLVKGFYPSDIAVEWESNGQPENNYKTTPPVLDSDGSFFLYSALTVDKSRWQQGNVFSCSVMHEALHNHYTQKSLSLSPGK

SEQ ID NO: 26 - DNA, 1227 bp, synthetic construct
  source 1..1227: mol_type = other DNA
tgcgatttaccccagacacactctttaggctctcgtaggaccctcatgctgctggcccagatgaggaggatctctttattctcttgtttaaaggacagacacgacttcggcttcccccaagaagagttcggcaaccagttccagaaggctgagaccatccccgtgctgcacgagatgatccagcagatcttcaatttatttagcaccaaggactccagcgccgcttgggatgagactttactggacaagttctacaccgaactgtaccagcagctgaacgatttagaggcttgtgtgatccaaggtgtgggagtgaccgagacccctctgatgaaggaggactccattttagccgtgaggaagtactttcgtaggatcaccctctacctcaaggagaagaagtacagcccttgcgcttgggaggtggtgagggctgagattatgaggagcttctctttatccaccaatctgcaagaatctttaaggtccaaggaaggcggaggcggatcaggcggcggtggatctgggggtggcggatctcgtacggacaaaacccacacatgcccaccttgtcccgcccctgaagccgcaggcggaccgtcagtcttcctcttccccccaaaacccaaggacaccctcatgatctcccggacccctgaggtcacatgcgtggtggtggacgtgagccacgaagaccctgaggtcaagttcaactggtacgtggacggcgtggaggtgcataatgccaagacaaagccgcgggaggagcagtacaacagcacgtaccgtgtggtcagcgtcctcaccgtcctgcaccaggactggctgaatggcaaggagtacaagtgcaaggtctccaacaaagccctcggagcccccatcgagaaaaccatctccaaagccaaagggcagccccgagaaccacaggtgtacaccctgcccccatgtcgggatgagctgaccaagaaccaggtcagcctgtggtgcctggtcaaaggcttctatcccagcgacatcgccgtggagtgggagagcaatgggcagccggagaacaactacaagaccacgcctcccgtgttggactccgacggctccttcttcctctacagcgcgctcaccgtggacaagagcaggtggcagcaggggaacgtcttctcatgctccgtgatgcatgaggctctgcacaaccactacacgcagaagagcctctccctgtctccgggtaaa